European Patent Specification EP 3 518 667 B1, published October 30, 2024. Title: NON-HUMAN ANIMALS HAVING A HEXANUCLEOTIDE REPEAT EXPANSION IN A C9ORF72 LOCUS. Applicant: Regeneron Pharmaceuticals, Inc Heslin, David Ally, Roxanne Siao, Chia-Jen Lai, Ka-Man Venus Valenzuela, David M. Guo, Chunguang LaCroix-Fralish, Michael Macdonald, Lynn Sharma, Aarti Kajimura, Daisuke Droguett, Gustavo Frendewey, David. The sequence listing filed with the application follows.

SEQUENCE LISTING (84 sequences)

SEQ ID NO: 1 - DNA, 6 bp, Artificial Sequence
  Heterologous Hexanucleotide sequence
ggggcc

SEQ ID NO: 2 - DNA, 964 bp, Homo sapiens
gggtctagcaagagcaggtgtgggtttaggaggtgtgtgtttttgtttttcccaccctctctccccactacttgctctcacagtactcgctgagggtgaacaagaaaagacctgataaagattaaccagaagaaaacaaggagggaaacaaccgcagcctgtagcaagctctggaactcaggagtcgcgcgctatgcgatcgcggggccggggccggggccgcgatcgcggggcgtggtcggggcgggcccgggggcgggcccggggcggggctgcggttgcggtgcctgcgcccgcggcggcggaggcgcaggcggtggcgagtgggtgagtgaggaggcggcatcctggcgggtggctgtttggggttcggctgccgggaagaggcgcgggtagaagcgggggctctcctcagagctcgacgcatttttactttccctctcatttctctgaccgaagctgggtgtcgggctttcgcctctagcgactggtggaattgcctgcatccgggccccgggcttcccggcggcggcggcggcggcggcggcgcagggacaagggatggggatctggcctcttccttgctttcccgccctcagtacccgagctgtctccttcccggggacccgctgggagcgctgccgctgcgggctcgagaaaagggagcctcgggtactgagaggcctcgcctgggggaaggccggagggtgggcggcgcgcggcttctgcggaccaagtcggggttcgctaggaacccgagacggtccctgccggcgaggagatcatgcgggatgagatgggggtgtggagacgcctgcacaatttcagcccaagcttctagagagtggtgatgacttgcatatgagggcagcaatgcaagtcggtgtgctccccattctgtgggacatgacctggttgcttcacagctccgagatgacacagacttgcttaaaggaagtgactc

SEQ ID NO: 3 - DNA, 1528 bp, Homo sapiens
gggtctagcaagagcaggtgtgggtttaggaggtgtgtgtttttgtttttcccaccctctctccccactacttgctctcacagtactcgctgagggtgaacaagaaaagacctgataaagattaaccagaagaaaacaaggagggaaacaaccgcagcctgtagcaagctctggaactcaggagtcgcgcgctatgcgatcgccgtctcggggccggggccggggccggggccggggccggggccggggccggggccggggccggggccggggccggggccggggccggggccggggccggggccggggccggggccggggccggggccggggccggggccggggccggggccggggccggggccggggccggggccggggccggggccggggccggggccggggccggggccggggccggggccggggccggggccggggccggggccggggccggggccggggccggggccggggccggggccggggccggggccggggccggggccggggccggggccggggccggggccggggccggggccggggccggggccggggccggggccggggccggggccggggccggggccggggccggggccggggccggggccggggccggggccggggccggggccggggccggggccggggccggggccggggccggggccggggccggggccggggccggggccggggccggggccggggccggggccggggccggggccggggccggggccggggccggggccgagaccctcgagggccggccgctagcgcgatcgcggggcgtggtcggggcgggcccgggggcgggcccggggcggggctgcggttgcggtgcctgcgcccgcggcggcggaggcgcaggcggtggcgagtgggtgagtgaggaggcggcatcctggcgggtggctgtttggggttcggctgccgggaagaggcgcgggtagaagcgggggctctcctcagagctcgacgcatttttactttccctctcatttctctgaccgaagctgggtgtcgggctttcgcctctagcgactggtggaattgcctgcatccgggccccgggcttcccggcggcggcggcggcggcggcggcgcagggacaagggatggggatctggcctcttccttgctttcccgccctcagtacccgagctgtctccttcccggggacccgctgggagcgctgccgctgcgggctcgagaaaagggagcctcgggtactgagaggcctcgcctgggggaaggccggagggtgggcggcgcgcggcttctgcggaccaagtcggggttcgctaggaacccgagacggtccctgccggcgaggagatcatgcgggatgagatgggggtgtggagacgcctgcacaatttcagcccaagcttctagagagtggtgatgacttgcatatgagggcagcaatgcaagtcggtgtgctccccattctgtgggacatgacctggttgcttcacagctccgagatgacacagacttgcttaaaggaagtgac

SEQ ID NO: 4 - DNA, 3621 bp, Artificial Sequence
  8026 insert nucleic acid without homology arms
gggtctagcaagagcaggtgtgggtttaggaggtgtgtgtttttgtttttcccaccctctctccccactacttgctctcacagtactcgctgagggtgaacaagaaaagacctgataaagattaaccagaagaaaacaaggagggaaacaaccgcagcctgtagcaagctctggaactcaggagtcgcgcgctatgcgatcgcggggccggggccggggccgcgatcgcggggcgtggtcggggcgggcccgggggcgggcccggggcggggctgcggttgcggtgcctgcgcccgcggcggcggaggcgcaggcggtggcgagtgggtgagtgaggaggcggcatcctggcgggtggctgtttggggttcggctgccgggaagaggcgcgggtagaagcgggggctctcctcagagctcgacgcatttttactttccctctcatttctctgaccgaagctgggtgtcgggctttcgcctctagcgactggtggaattgcctgcatccgggccccgggcttcccggcggcggcggcggcggcggcggcgcagggacaagggatggggatctggcctcttccttgctttcccgccctcagtacccgagctgtctccttcccggggacccgctgggagcgctgccgctgcgggctcgagaaaagggagcctcgggtactgagaggcctcgcctgggggaaggccggagggtgggcggcgcgcggcttctgcggaccaagtcggggttcgctaggaacccgagacggtccctgccggcgaggagatcatgcgggatgagatgggggtgtggagacgcctgcacaatttcagcccaagcttctagagagtggtgatgacttgcatatgagggcagcaatgcaagtcggtgtgctccccattctgtgggacatgacctggttgcttcacagctccgagatgacacagacttgcttaaaggaagtgactcgagataacttcgtataatgtatgctatacgaagttatatgcatggcctccgcgccgggttttggcgcctcccgcgggcgcccccctcctcacggcgagcgctgccacgtcagacgaagggcgcagcgagcgtcctgatccttccgcccggacgctcaggacagcggcccgctgctcataagactcggccttagaaccccagtatcagcagaaggacattttaggacgggacttgggtgactctagggcactggttttctttccagagagcggaacaggcgaggaaaagtagtcccttctcggcgattctgcggagggatctccgtggggcggtgaacgccgatgattatataaggacgcgccgggtgtggcacagctagttccgtcgcagccgggatttgggtcgcggttcttgtttgtggatcgctgtgatcgtcacttggtgagtagcgggctgctgggctggccggggctttcgtggccgccgggccgctcggtgggacggaagcgtgtggagagaccgccaagggctgtagtctgggtccgcgagcaaggttgccctgaactgggggttggggggagcgcagcaaaatggcggctgttcccgagtcttgaatggaagacgcttgtgaggcgggctgtgaggtcgttgaaacaaggtggggggcatggtgggcggcaagaacccaaggtcttgaggccttcgctaatgcgggaaagctcttattcgggtgagatgggctggggcaccatctggggaccctgacgtgaagtttgtcactgactggagaactcggtttgtcgtctgttgcgggggcggcagttatggcggtgccgttgggcagtgcacccgtacctttgggagcgcgcgccctcgtcgtgtcgtgacgtcacccgttctgttggcttataatgcagggtggggccacctgccggtaggtgtgcggtaggcttttctccgtcgcaggacgcagggttcgggcctagggtaggctctcctgaatcgacaggcgccggacctctggtgaggggagggataagtgaggcgtcagtttctttggtcggttttatgtacctatcttcttaagtagctgaagctccggttttgaactatgcgctcggggttggcgagtgtgttttgtgaagttttttaggcaccttttgaaatgtaatcatttgggtcaatatgtaattttcagtgttagactagtaaattgtccgctaaattctggccgtttttggcttttttgttagacgtgttgacaattaatcatcggcatagtatatcggcatagtataatacgacaaggtgaggaactaaaccatgggatcggccattgaacaagatggattgcacgcaggttctccggccgcttgggtggagaggctattcggctatgactgggcacaacagacaatcggctgctctgatgccgccgtgttccggctgtcagcgcaggggcgcccggttctttttgtcaagaccgacctgtccggtgccctgaatgaactgcaggacgaggcagcgcggctatcgtggctggccacgacgggcgttccttgcgcagctgtgctcgacgttgtcactgaagcgggaagggactggctgctattgggcgaagtgccggggcaggatctcctgtcatctcaccttgctcctgccgagaaagtatccatcatggctgatgcaatgcggcggctgcatacgcttgatccggctacctgcccattcgaccaccaagcgaaacatcgcatcgagcgagcacgtactcggatggaagccggtcttgtcgatcaggatgatctggacgaagagcatcaggggctcgcgccagccgaactgttcgccaggctcaaggcgcgcatgcccgacggcgatgatctcgtcgtgacccatggcgatgcctgcttgccgaatatcatggtggaaaatggccgcttttctggattcatcgactgtggccggctgggtgtggcggaccgctatcaggacatagcgttggctacccgtgatattgctgaagagcttggcggcgaatgggctgaccgcttcctcgtgctttacggtatcgccgctcccgattcgcagcgcatcgccttctatcgccttcttgacgagttcttctgaggggatccgctgtaagtctgcagaaattgatgatctattaaacaataaagatgtccactaaaatggaagtttttcctgtcatactttgttaagaagggtgagaacagagtacctacattttgaatggaaggattggagctacgggggtgggggtggggtgggattagataaatgcctgctctttactgaaggctctttactattgctttatgataatgtttcatagttggatatcataatttaaacaagcaaaaccaaattaagggccagctcattcctcccactcatgatctatagatctatagatctctcgtgggatcattgtttttctcttgattcccactttgtggttctaagtactgtggtttccaaatgtgtcagtttcatagcctgaagaacgagatcagcagcctctgttccacatacacttcattctcagtattgttttgccaagttctaattccatcagacctcgacctgcagcccctagataacttcgtataatgtatgctatacgaagttatgctagc

SEQ ID NO: 5 - DNA, 1006 bp, Artificial Sequence
  8026 insert nucleic acid without homology arms and after excision of neo
gggtctagcaagagcaggtgtgggtttaggaggtgtgtgtttttgtttttcccaccctctctccccactacttgctctcacagtactcgctgagggtgaacaagaaaagacctgataaagattaaccagaagaaaacaaggagggaaacaaccgcagcctgtagcaagctctggaactcaggagtcgcgcgctatgcgatcgcggggccggggccggggccgcgatcgcggggcgtggtcggggcgggcccgggggcgggcccggggcggggctgcggttgcggtgcctgcgcccgcggcggcggaggcgcaggcggtggcgagtgggtgagtgaggaggcggcatcctggcgggtggctgtttggggttcggctgccgggaagaggcgcgggtagaagcgggggctctcctcagagctcgacgcatttttactttccctctcatttctctgaccgaagctgggtgtcgggctttcgcctctagcgactggtggaattgcctgcatccgggccccgggcttcccggcggcggcggcggcggcggcggcgcagggacaagggatggggatctggcctcttccttgctttcccgccctcagtacccgagctgtctccttcccggggacccgctgggagcgctgccgctgcgggctcgagaaaagggagcctcgggtactgagaggcctcgcctgggggaaggccggagggtgggcggcgcgcggcttctgcggaccaagtcggggttcgctaggaacccgagacggtccctgccggcgaggagatcatgcgggatgagatgggggtgtggagacgcctgcacaatttcagcccaagcttctagagagtggtgatgacttgcatatgagggcagcaatgcaagtcggtgtgctccccattctgtgggacatgacctggttgcttcacagctccgagatgacacagacttgcttaaaggaagtgactcgagataacttcgtataatgtatgctatacgaagttatgctag

SEQ ID NO: 6 - DNA, 4180 bp, Artificial Sequence
  8026 Insert Nucleic acid without homology arms plus neo cassette
ggtctagcaagagcaggtgtgggtttaggaggtgtgtgtttttgtttttcccaccctctctccccactacttgctctcacagtactcgctgagggtgaacaagaaaagacctgataaagattaaccagaagaaaacaaggagggaaacaaccgcagcctgtagcaagctctggaactcaggagtcgcgcgctatgcgatcgccgtctcggggccggggccggggccggggccggggccggggccggggccggggccggggccggggccggggccggggccggggccggggccggggccggggccggggccggggccggggccggggccggggccggggccggggccggggccggggccggggccggggccggggccggggccggggccggggccggggccggggccggggccggggccggggccggggccggggccggggccggggccggggccggggccggggccggggccggggccggggccggggccggggccggggccggggccggggccggggccggggccggggccggggccggggccggggccggggccggggccggggccggggccggggccggggccggggccggggccggggccggggccggggccggggccggggccggggccggggccggggccggggccggggccggggccggggccggggccggggccggggccggggccggggccggggccggggccggggccggggccggggccggggccggggccggggccggggccggggccgagaccctcgagggccggccgctagcgcgatcgcggggcgtggtcggggcgggcccgggggcgggcccggggcggggctgcggttgcggtgcctgcgcccgcggcggcggaggcgcaggcggtggcgagtgggtgagtgaggaggcggcatcctggcgggtggctgtttggggttcggctgccgggaagaggcgcgggtagaagcgggggctctcctcagagctcgacgcatttttactttccctctcatttctctgaccgaagctgggtgtcgggctttcgcctctagcgactggtggaattgcctgcatccgggccccgggcttcccggcggcggcggcggcggcggcggcgcagggacaagggatggggatctggcctcttccttgctttcccgccctcagtacccgagctgtctccttcccggggacccgctgggagcgctgccgctgcgggctcgagaaaagggagcctcgggtactgagaggcctcgcctgggggaaggccggagggtgggcggcgcgcggcttctgcggaccaagtcggggttcgctaggaacccgagacggtccctgccggcgaggagatcatgcgggatgagatgggggtgtggagacgcctgcacaatttcagcccaagcttctagagagtggtgatgacttgcatatgagggcagcaatgcaagtcggtgtgctccccattctgtgggacatgacctggttgcttcacagctccgagatgacacagacttgcttaaaggaagtgactcgagataacttcgtataatgtatgctatacgaagttatatgcatggcctccgcgccgggttttggcgcctcccgcgggcgcccccctcctcacggcgagcgctgccacgtcagacgaagggcgcagcgagcgtcctgatccttccgcccggacgctcaggacagcggcccgctgctcataagactcggccttagaaccccagtatcagcagaaggacattttaggacgggacttgggtgactctagggcactggttttctttccagagagcggaacaggcgaggaaaagtagtcccttctcggcgattctgcggagggatctccgtggggcggtgaacgccgatgattatataaggacgcgccgggtgtggcacagctagttccgtcgcagccgggatttgggtcgcggttcttgtttgtggatcgctgtgatcgtcacttggtgagtagcgggctgctgggctggccggggctttcgtggccgccgggccgctcggtgggacggaagcgtgtggagagaccgccaagggctgtagtctgggtccgcgagcaaggttgccctgaactgggggttggggggagcgcagcaaaatggcggctgttcccgagtcttgaatggaagacgcttgtgaggcgggctgtgaggtcgttgaaacaaggtggggggcatggtgggcggcaagaacccaaggtcttgaggccttcgctaatgcgggaaagctcttattcgggtgagatgggctggggcaccatctggggaccctgacgtgaagtttgtcactgactggagaactcggtttgtcgtctgttgcgggggcggcagttatggcggtgccgttgggcagtgcacccgtacctttgggagcgcgcgccctcgtcgtgtcgtgacgtcacccgttctgttggcttataatgcagggtggggccacctgccggtaggtgtgcggtaggcttttctccgtcgcaggacgcagggttcgggcctagggtaggctctcctgaatcgacaggcgccggacctctggtgaggggagggataagtgaggcgtcagtttctttggtcggttttatgtacctatcttcttaagtagctgaagctccggttttgaactatgcgctcggggttggcgagtgtgttttgtgaagttttttaggcaccttttgaaatgtaatcatttgggtcaatatgtaattttcagtgttagactagtaaattgtccgctaaattctggccgtttttggcttttttgttagacgtgttgacaattaatcatcggcatagtatatcggcatagtataatacgacaaggtgaggaactaaaccatgggatcggccattgaacaagatggattgcacgcaggttctccggccgcttgggtggagaggctattcggctatgactgggcacaacagacaatcggctgctctgatgccgccgtgttccggctgtcagcgcaggggcgcccggttctttttgtcaagaccgacctgtccggtgccctgaatgaactgcaggacgaggcagcgcggctatcgtggctggccacgacgggcgttccttgcgcagctgtgctcgacgttgtcactgaagcgggaagggactggctgctattgggcgaagtgccggggcaggatctcctgtcatctcaccttgctcctgccgagaaagtatccatcatggctgatgcaatgcggcggctgcatacgcttgatccggctacctgcccattcgaccaccaagcgaaacatcgcatcgagcgagcacgtactcggatggaagccggtcttgtcgatcaggatgatctggacgaagagcatcaggggctcgcgccagccgaactgttcgccaggctcaaggcgcgcatgcccgacggcgatgatctcgtcgtgacccatggcgatgcctgcttgccgaatatcatggtggaaaatggccgcttttctggattcatcgactgtggccggctgggtgtggcggaccgctatcaggacatagcgttggctacccgtgatattgctgaagagcttggcggcgaatgggctgaccgcttcctcgtgctttacggtatcgccgctcccgattcgcagcgcatcgccttctatcgccttcttgacgagttcttctgaggggatccgctgtaagtctgcagaaattgatgatctattaaacaataaagatgtccactaaaatggaagtttttcctgtcatactttgttaagaagggtgagaacagagtacctacattttgaatggaaggattggagctacgggggtgggggtggggtgggattagataaatgcctgctctttactgaaggctctttactattgctttatgataatgtttcatagttggatatcataatttaaacaagcaaaaccaaattaagggccagctcattcctcccactcatgatctatagatctatagatctctcgtgggatcattgtttttctcttgattcccactttgtggttctaagtactgtggtttccaaatgtgtcagtttcatagcctgaagaacgagatcagcagcctctgttccacatacacttcattctcagtattgttttgccaagttctaattccatcagacctcgacctgcagcccctagataacttcgtataatgtatgctatacgaagttat

SEQ ID NO: 7 - DNA, 1566 bp, Artificial Sequence
  8028 insert nucleic acid with lox site after excision of neo and without homology arms
gggtctagcaagagcaggtgtgggtttaggaggtgtgtgtttttgtttttcccaccctctctccccactacttgctctcacagtactcgctgagggtgaacaagaaaagacctgataaagattaaccagaagaaaacaaggagggaaacaaccgcagcctgtagcaagctctggaactcaggagtcgcgcgctatgcgatcgccgtctcggggccggggccggggccggggccggggccggggccggggccggggccggggccggggccggggccggggccggggccggggccggggccggggccggggccggggccggggccggggccggggccggggccggggccggggccggggccggggccggggccggggccggggccggggccggggccggggccggggccggggccggggccggggccggggccggggccggggccggggccggggccggggccggggccggggccggggccggggccggggccggggccggggccggggccggggccggggccggggccggggccggggccggggccggggccggggccggggccggggccggggccggggccggggccggggccggggccggggccggggccggggccggggccggggccggggccggggccggggccggggccggggccggggccggggccggggccggggccggggccggggccggggccggggccggggccggggccggggccggggccggggccggggccggggccggggccggggccgagaccctcgagggccggccgctagcgcgatcgcggggcgtggtcggggcgggcccgggggcgggcccggggcggggctgcggttgcggtgcctgcgcccgcggcggcggaggcgcaggcggtggcgagtgggtgagtgaggaggcggcatcctggcgggtggctgtttggggttcggctgccgggaagaggcgcgggtagaagcgggggctctcctcagagctcgacgcatttttactttccctctcatttctctgaccgaagctgggtgtcgggctttcgcctctagcgactggtggaattgcctgcatccgggccccgggcttcccggcggcggcggcggcggcggcggcgcagggacaagggatggggatctggcctcttccttgctttcccgccctcagtacccgagctgtctccttcccggggacccgctgggagcgctgccgctgcgggctcgagaaaagggagcctcgggtactgagaggcctcgcctgggggaaggccggagggtgggcggcgcgcggcttctgcggaccaagtcggggttcgctaggaacccgagacggtccctgccggcgaggagatcatgcgggatgagatgggggtgtggagacgcctgcacaatttcagcccaagcttctagagagtggtgatgacttgcatatgagggcagcaatgcaagtcggtgtgctccccattctgtgggacatgacctggttgcttcacagctccgagatgacacagacttgcttaaaggaagtgactcgagataacttcgtataatgtatgctatacgaagtta

SEQ ID NO: 8 - DNA, 3821 bp, Artificial Sequence
  8026 targeting nucleic acid with homology arms and neo cassette
gaaccgcggcgcgtcaagcagagacgagttccgcccacgtgaaagatggcgtttgtagtgacagccatcccaattgccctttccttctaggtggaaagtggggtctagcaagagcaggtgtgggtttaggaggtgtgtgtttttgtttttcccaccctctctccccactacttgctctcacagtactcgctgagggtgaacaagaaaagacctgataaagattaaccagaagaaaacaaggagggaaacaaccgcagcctgtagcaagctctggaactcaggagtcgcgcgctatgcgatcgcggggccggggccggggccgcgatcgcggggcgtggtcggggcgggcccgggggcgggcccggggcggggctgcggttgcggtgcctgcgcccgcggcggcggaggcgcaggcggtggcgagtgggtgagtgaggaggcggcatcctggcgggtggctgtttggggttcggctgccgggaagaggcgcgggtagaagcgggggctctcctcagagctcgacgcatttttactttccctctcatttctctgaccgaagctgggtgtcgggctttcgcctctagcgactggtggaattgcctgcatccgggccccgggcttcccggcggcggcggcggcggcggcggcgcagggacaagggatggggatctggcctcttccttgctttcccgccctcagtacccgagctgtctccttcccggggacccgctgggagcgctgccgctgcgggctcgagaaaagggagcctcgggtactgagaggcctcgcctgggggaaggccggagggtgggcggcgcgcggcttctgcggaccaagtcggggttcgctaggaacccgagacggtccctgccggcgaggagatcatgcgggatgagatgggggtgtggagacgcctgcacaatttcagcccaagcttctagagagtggtgatgacttgcatatgagggcagcaatgcaagtcggtgtgctccccattctgtgggacatgacctggttgcttcacagctccgagatgacacagacttgcttaaaggaagtgactcgagataacttcgtataatgtatgctatacgaagttatatgcatggcctccgcgccgggttttggcgcctcccgcgggcgcccccctcctcacggcgagcgctgccacgtcagacgaagggcgcagcgagcgtcctgatccttccgcccggacgctcaggacagcggcccgctgctcataagactcggccttagaaccccagtatcagcagaaggacattttaggacgggacttgggtgactctagggcactggttttctttccagagagcggaacaggcgaggaaaagtagtcccttctcggcgattctgcggagggatctccgtggggcggtgaacgccgatgattatataaggacgcgccgggtgtggcacagctagttccgtcgcagccgggatttgggtcgcggttcttgtttgtggatcgctgtgatcgtcacttggtgagtagcgggctgctgggctggccggggctttcgtggccgccgggccgctcggtgggacggaagcgtgtggagagaccgccaagggctgtagtctgggtccgcgagcaaggttgccctgaactgggggttggggggagcgcagcaaaatggcggctgttcccgagtcttgaatggaagacgcttgtgaggcgggctgtgaggtcgttgaaacaaggtggggggcatggtgggcggcaagaacccaaggtcttgaggccttcgctaatgcgggaaagctcttattcgggtgagatgggctggggcaccatctggggaccctgacgtgaagtttgtcactgactggagaactcggtttgtcgtctgttgcgggggcggcagttatggcggtgccgttgggcagtgcacccgtacctttgggagcgcgcgccctcgtcgtgtcgtgacgtcacccgttctgttggcttataatgcagggtggggccacctgccggtaggtgtgcggtaggcttttctccgtcgcaggacgcagggttcgggcctagggtaggctctcctgaatcgacaggcgccggacctctggtgaggggagggataagtgaggcgtcagtttctttggtcggttttatgtacctatcttcttaagtagctgaagctccggttttgaactatgcgctcggggttggcgagtgtgttttgtgaagttttttaggcaccttttgaaatgtaatcatttgggtcaatatgtaattttcagtgttagactagtaaattgtccgctaaattctggccgtttttggcttttttgttagacgtgttgacaattaatcatcggcatagtatatcggcatagtataatacgacaaggtgaggaactaaaccatgggatcggccattgaacaagatggattgcacgcaggttctccggccgcttgggtggagaggctattcggctatgactgggcacaacagacaatcggctgctctgatgccgccgtgttccggctgtcagcgcaggggcgcccggttctttttgtcaagaccgacctgtccggtgccctgaatgaactgcaggacgaggcagcgcggctatcgtggctggccacgacgggcgttccttgcgcagctgtgctcgacgttgtcactgaagcgggaagggactggctgctattgggcgaagtgccggggcaggatctcctgtcatctcaccttgctcctgccgagaaagtatccatcatggctgatgcaatgcggcggctgcatacgcttgatccggctacctgcccattcgaccaccaagcgaaacatcgcatcgagcgagcacgtactcggatggaagccggtcttgtcgatcaggatgatctggacgaagagcatcaggggctcgcgccagccgaactgttcgccaggctcaaggcgcgcatgcccgacggcgatgatctcgtcgtgacccatggcgatgcctgcttgccgaatatcatggtggaaaatggccgcttttctggattcatcgactgtggccggctgggtgtggcggaccgctatcaggacatagcgttggctacccgtgatattgctgaagagcttggcggcgaatgggctgaccgcttcctcgtgctttacggtatcgccgctcccgattcgcagcgcatcgccttctatcgccttcttgacgagttcttctgaggggatccgctgtaagtctgcagaaattgatgatctattaaacaataaagatgtccactaaaatggaagtttttcctgtcatactttgttaagaagggtgagaacagagtacctacattttgaatggaaggattggagctacgggggtgggggtggggtgggattagataaatgcctgctctttactgaaggctctttactattgctttatgataatgtttcatagttggatatcataatttaaacaagcaaaaccaaattaagggccagctcattcctcccactcatgatctatagatctatagatctctcgtgggatcattgtttttctcttgattcccactttgtggttctaagtactgtggtttccaaatgtgtcagtttcatagcctgaagaacgagatcagcagcctctgttccacatacacttcattctcagtattgttttgccaagttctaattccatcagacctcgacctgcagcccctagataacttcgtataatgtatgctatacgaagttatgctagcattgtgacttgggcatcacttgactgatggtaatcagttgcagagagagaagtgcactgattaagtctgtccacacagggtctgtctggccaggagtgca

SEQ ID NO: 9 - DNA, 4387 bp, Artificial Sequence
  8026 insert nucleic acid with homology arms, hexanucleotide repeat(s) and neo cassette
gaaccgcggcgcgtcaagcagagacgagttccgcccacgtgaaagatggcgtttgtagtgacagccatcccaattgccctttccttctaggtggaaagtggggtctagcaagagcaggtgtgggtttaggaggtgtgtgtttttgtttttcccaccctctctccccactacttgctctcacagtactcgctgagggtgaacaagaaaagacctgataaagattaaccagaagaaaacaaggagggaaacaaccgcagcctgtagcaagctctggaactcaggagtcgcgcgctatgcgatcgccgtctcggggccggggccggggccggggccggggccggggccggggccggggccggggccggggccggggccggggccggggccggggccggggccggggccggggccggggccggggccggggccggggccggggccggggccggggccggggccggggccggggccggggccggggccggggccggggccggggccggggccggggccggggccggggccggggccggggccggggccggggccggggccggggccggggccggggccggggccggggccggggccggggccggggccggggccggggccggggccggggccggggccggggccggggccggggccggggccggggccggggccggggccggggccggggccggggccggggccggggccggggccggggccggggccggggccggggccggggccggggccggggccggggccggggccggggccggggccggggccggggccggggccggggccggggccggggccggggccggggccggggccggggccggggccggggccggggccggggccgagaccctcgagggccggccgctagcgcgatcgcggggcgtggtcggggcgggcccgggggcgggcccggggcggggctgcggttgcggtgcctgcgcccgcggcggcggaggcgcaggcggtggcgagtgggtgagtgaggaggcggcatcctggcgggtggctgtttggggttcggctgccgggaagaggcgcgggtagaagcgggggctctcctcagagctcgacgcatttttactttccctctcatttctctgaccgaagctgggtgtcgggctttcgcctctagcgactggtggaattgcctgcatccgggccccgggcttcccggcggcggcggcggcggcggcggcgcagggacaagggatggggatctggcctcttccttgctttcccgccctcagtacccgagctgtctccttcccggggacccgctgggagcgctgccgctgcgggctcgagaaaagggagcctcgggtactgagaggcctcgcctgggggaaggccggagggtgggcggcgcgcggcttctgcggaccaagtcggggttcgctaggaacccgagacggtccctgccggcgaggagatcatgcgggatgagatgggggtgtggagacgcctgcacaatttcagcccaagcttctagagagtggtgatgacttgcatatgagggcagcaatgcaagtcggtgtgctccccattctgtgggacatgacctggttgcttcacagctccgagatgacacagacttgcttaaaggaagtgactcgagataacttcgtataatgtatgctatacgaagttatatgcatggcctccgcgccgggttttggcgcctcccgcgggcgcccccctcctcacggcgagcgctgccacgtcagacgaagggcgcagcgagcgtcctgatccttccgcccggacgctcaggacagcggcccgctgctcataagactcggccttagaaccccagtatcagcagaaggacattttaggacgggacttgggtgactctagggcactggttttctttccagagagcggaacaggcgaggaaaagtagtcccttctcggcgattctgcggagggatctccgtggggcggtgaacgccgatgattatataaggacgcgccgggtgtggcacagctagttccgtcgcagccgggatttgggtcgcggttcttgtttgtggatcgctgtgatcgtcacttggtgagtagcgggctgctgggctggccggggctttcgtggccgccgggccgctcggtgggacggaagcgtgtggagagaccgccaagggctgtagtctgggtccgcgagcaaggttgccctgaactgggggttggggggagcgcagcaaaatggcggctgttcccgagtcttgaatggaagacgcttgtgaggcgggctgtgaggtcgttgaaacaaggtggggggcatggtgggcggcaagaacccaaggtcttgaggccttcgctaatgcgggaaagctcttattcgggtgagatgggctggggcaccatctggggaccctgacgtgaagtttgtcactgactggagaactcggtttgtcgtctgttgcgggggcggcagttatggcggtgccgttgggcagtgcacccgtacctttgggagcgcgcgccctcgtcgtgtcgtgacgtcacccgttctgttggcttataatgcagggtggggccacctgccggtaggtgtgcggtaggcttttctccgtcgcaggacgcagggttcgggcctagggtaggctctcctgaatcgacaggcgccggacctctggtgaggggagggataagtgaggcgtcagtttctttggtcggttttatgtacctatcttcttaagtagctgaagctccggttttgaactatgcgctcggggttggcgagtgtgttttgtgaagttttttaggcaccttttgaaatgtaatcatttgggtcaatatgtaattttcagtgttagactagtaaattgtccgctaaattctggccgtttttggcttttttgttagacgtgttgacaattaatcatcggcatagtatatcggcatagtataatacgacaaggtgaggaactaaaccatgggatcggccattgaacaagatggattgcacgcaggttctccggccgcttgggtggagaggctattcggctatgactgggcacaacagacaatcggctgctctgatgccgccgtgttccggctgtcagcgcaggggcgcccggttctttttgtcaagaccgacctgtccggtgccctgaatgaactgcaggacgaggcagcgcggctatcgtggctggccacgacgggcgttccttgcgcagctgtgctcgacgttgtcactgaagcgggaagggactggctgctattgggcgaagtgccggggcaggatctcctgtcatctcaccttgctcctgccgagaaagtatccatcatggctgatgcaatgcggcggctgcatacgcttgatccggctacctgcccattcgaccaccaagcgaaacatcgcatcgagcgagcacgtactcggatggaagccggtcttgtcgatcaggatgatctggacgaagagcatcaggggctcgcgccagccgaactgttcgccaggctcaaggcgcgcatgcccgacggcgatgatctcgtcgtgacccatggcgatgcctgcttgccgaatatcatggtggaaaatggccgcttttctggattcatcgactgtggccggctgggtgtggcggaccgctatcaggacatagcgttggctacccgtgatattgctgaagagcttggcggcgaatgggctgaccgcttcctcgtgctttacggtatcgccgctcccgattcgcagcgcatcgccttctatcgccttcttgacgagttcttctgaggggatccgctgtaagtctgcagaaattgatgatctattaaacaataaagatgtccactaaaatggaagtttttcctgtcatactttgttaagaagggtgagaacagagtacctacattttgaatggaaggattggagctacgggggtgggggtggggtgggattagataaatgcctgctctttactgaaggctctttactattgctttatgataatgtttcatagttggatatcataatttaaacaagcaaaaccaaattaagggccagctcattcctcccactcatgatctatagatctatagatctctcgtgggatcattgtttttctcttgattcccactttgtggttctaagtactgtggtttccaaatgtgtcagtttcatagcctgaagaacgagatcagcagcctctgttccacatacacttcattctcagtattgttttgccaagttctaattccatcagacctcgacctgcagcccctagataacttcgtataatgtatgctatacgaagttatgctagcattgtgacttgggcatcacttgactgatggtaatcagttgcagagagagaagtgcactgattaagtctgtccacacagggtctgtctggccaggagtgca

SEQ ID NO: 10 - DNA, 1957 bp, Homo sapiens
acgtaacctacggtgtcccgctaggaaagagaggtgcgtcaaacagcgacaagttccgcccacgtaaaagatgacgcttgatatctccggagcatttggataatgtgacagttggaatgcagtgatgtcgactctttgcccaccgccatctccagctgttgccaagacagagattgctttaagtggcaaatcacctttattagcagctacttttgcttactgggacaatattcttggtcctagagtaaggcacatttgggctccaaagacagaacaggtacttctcagtgatggagaaataacttttcttgccaaccacactctaaatggagaaatccttcgaaatgcagagagtggtgctatagatgtaaagttttttgtcttgtctgaaaagggagtgattattgtttcattaatctttgatggaaactggaatggggatcgcagcacatatggactatcaattatacttccacagacagaacttagtttctacctcccacttcatagagtgtgtgttgatagattaacacatataatccggaaaggaagaatatggatgcataaggaaagacaagaaaatgtccagaagattatcttagaaggcacagagagaatggaagatcagggtcagagtattattccaatgcttactggagaagtgattcctgtaatggaactgctttcatctatgaaatcacacagtgttcctgaagaaatagatatagctgatacagtactcaatgatgatgatattggtgacagctgtcatgaaggctttcttctcaagtaagaatttttcttttcataaaagctggatgaagcagataccatcttatgctcacctatgacaagatttggaagaaagaaaataacagactgtctacttagattgttctagggacattacgtatttgaactgttgcttaaatttgtgttatttttcactcattatatttctatatatatttggtgttattccatttgctatttaaagaaaccgagtttccatcccagacaagaaatcatggccccttgcttgattctggtttcttgttttacttctcattaaagctaacagaatcctttcatattaagttgtactgtagatgaacttaagttatttaggcgtagaacaaaattattcatatttatactgatctttttccatccagcagtggagtttagtacttaagagtttgtgcccttaaaccagactccctggattaatgctgtgtacccgtgggcaaggtgcctgaattctctatacacctatttcctcatctgtaaaatggcaataatagtaatagtacctaatgtgtagggttgttataagcattgagtaagataaataatataaagcacttagaacagtgcctggaacataaaaacacttaataatagctcatagctaacatttcctatttacatttcttctagaaatagccagtatttgttgagtgcctacatgttagttcctttactagttgctttacatgtattatcttatattctgttttaaagtttcttcacagttacagattttcatgaaattttacttttaataaaagagaagtaaaagtataaagtattcacttttatgttcacagtcttttcctttaggctcatgatggagtatcagaggcatgagtgtgtttaacctaagagccttaatggcttgaatcagaagcactttagtcctgtatctgttcagtgtcagcctttcatacatcattttaaatcccatttgactttaagtaagtcacttaatctctctacatgtcaatttcttcagctataaaatgatggtatttcaataaataaatacattaattaaatgatattatactgactaattgggctgttttaaggctcaataagaaaatttctgtgaaaggtctctagaaaatgtaggttcctatacaaataaaagataacattgtgcttataaaaaaaa

SEQ ID NO: 11 - protein, 222 aa, Homo sapiens
MSTLCPPPSPAVAKTEIALSGKSPLLAATFAYWDNILGPRVRHIWAPKTEQVLLSDGEITFLANHTLNGEILRNAESGAIDVKFFVLSEKGVIIVSLIFDGNWNGDRSTYGLSIILPQTELSFYLPLHRVCVDRLTHIIRKGRIWMHKERQENVQKIILEGTERMEDQGQSIIPMLTGEVIPVMELLSSMKSHSVPEEIDIADTVLNDDDIGDSCHEGFLLK

SEQ ID NO: 12 - DNA, 3261 bp, Homo sapiens
gggcggggctgcggttgcggtgcctgcgcccgcggcggcggaggcgcaggcggtggcgagtggatatctccggagcatttggataatgtgacagttggaatgcagtgatgtcgactctttgcccaccgccatctccagctgttgccaagacagagattgctttaagtggcaaatcacctttattagcagctacttttgcttactgggacaatattcttggtcctagagtaaggcacatttgggctccaaagacagaacaggtacttctcagtgatggagaaataacttttcttgccaaccacactctaaatggagaaatccttcgaaatgcagagagtggtgctatagatgtaaagttttttgtcttgtctgaaaagggagtgattattgtttcattaatctttgatggaaactggaatggggatcgcagcacatatggactatcaattatacttccacagacagaacttagtttctacctcccacttcatagagtgtgtgttgatagattaacacatataatccggaaaggaagaatatggatgcataaggaaagacaagaaaatgtccagaagattatcttagaaggcacagagagaatggaagatcagggtcagagtattattccaatgcttactggagaagtgattcctgtaatggaactgctttcatctatgaaatcacacagtgttcctgaagaaatagatatagctgatacagtactcaatgatgatgatattggtgacagctgtcatgaaggctttcttctcaatgccatcagctcacacttgcaaacctgtggctgttccgttgtagtaggtagcagtgcagagaaagtaaataagatagtcagaacattatgcctttttctgactccagcagagagaaaatgctccaggttatgtgaagcagaatcatcatttaaatatgagtcagggctctttgtacaaggcctgctaaaggattcaactggaagctttgtgctgcctttccggcaagtcatgtatgctccatatcccaccacacacatagatgtggatgtcaatactgtgaagcagatgccaccctgtcatgaacatatttataatcagcgtagatacatgagatccgagctgacagccttctggagagccacttcagaagaagacatggctcaggatacgatcatctacactgacgaaagctttactcctgatttgaatatttttcaagatgtcttacacagagacactctagtgaaagccttcctggatcaggtctttcagctgaaacctggcttatctctcagaagtactttccttgcacagtttctacttgtccttcacagaaaagccttgacactaataaaatatatagaagacgatacgcagaagggaaaaaagccctttaaatctcttcggaacctgaagatagaccttgatttaacagcagagggcgatcttaacataataatggctctggctgagaaaattaaaccaggcctacactcttttatctttggaagacctttctacactagtgtgcaagaacgagatgttctaatgactttttaaatgtgtaacttaataagcctattccatcacaatcatgatcgctggtaaagtagctcagtggtgtggggaaacgttcccctggatcatactccagaattctgctctcagcaattgcagttaagtaagttacactacagttctcacaagagcctgtgaggggatgtcaggtgcatcattacattgggtgtctcttttcctagatttatgcttttgggatacagacctatgtttacaatataataaatattattgctatcttttaaagatataataataggatgtaaacttgaccacaactactgtttttttgaaatacatgattcatggtttacatgtgtcaaggtgaaatctgagttggcttttacagatagttgactttctatcttttggcattctttggtgtgtagaattactgtaatacttctgcaatcaactgaaaactagagcctttaaatgatttcaattccacagaaagaaagtgagcttgaacataggatgagctttagaaagaaaattgatcaagcagatgtttaattggaattgattattagatcctactttgtggatttagtccctgggattcagtctgtagaaatgtctaatagttctctatagtccttgttcctggtgaaccacagttagggtgttttgtttattttattgttcttgctattgttgatattctatgtagttgagctctgtaaaaggaaattgtattttatgttttagtaattgttgccaactttttaaattaattttcattatttttgagccaaattgaaatgtgcacctcctgtgccttttttctccttagaaaatctaattacttggaacaagttcagatttcactggtcagtcattttcatcttgttttcttcttgctaagtcttaccatgtacctgctttggcaatcattgcaactctgagattataaaatgccttagagaatatactaactaataagatctttttttcagaaacagaaaatagttccttgagtacttccttcttgcatttctgcctatgtttttgaagttgttgctgtttgcctgcaataggctataaggaatagcaggagaaattttactgaagtgctgttttcctaggtgctactttggcagagctaagttatcttttgttttcttaatgcgtttggaccattttgctggctataaaataactgattaatataattctaacacaatgttgacattgtagttacacaaacacaaataaatattttatttaaaattctggaagtaatataaaagggaaaatatatttataagaaagggataaaggtaatagagcccttctgccccccacccaccaaatttacacaacaaaatgacatgttcgaatgtgaaaggtcataatagctttcccatcatgaatcagaaagatgtggacagcttgatgttttagacaaccactgaactagatgactgttgtactgtagctcagtcatttaaaaaatatataaatactaccttgtagtgtcccatactgtgttttttacatggtagattcttatttaagtgctaactggttattttctttggctggtttattgtactgttatacagaatgtaagttgtacagtgaaataagttattaaagcatgtgtaaacattgttatatatcttttctcctaaatggagaattttgaataaaatatatttgaaattttaaaaaaaaaaaaaaaaaa

SEQ ID NO: 13 - protein, 481 aa, Homo sapiens
MSTLCPPPSPAVAKTEIALSGKSPLLAATFAYWDNILGPRVRHIWAPKTEQVLLSDGEITFLANHTLNGEILRNAESGAIDVKFFVLSEKGVIIVSLIFDGNWNGDRSTYGLSIILPQTELSFYLPLHRVCVDRLTHIIRKGRIWMHKERQENVQKIILEGTERMEDQGQSIIPMLTGEVIPVMELLSSMKSHSVPEEIDIADTVLNDDDIGDSCHEGFLLNAISSHLQTCGCSVVVGSSAEKVNKIVRTLCLFLTPAERKCSRLCEAESSFKYESGLFVQGLLKDSTGSFVLPFRQVMYAPYPTTHIDVDVNTVKQMPPCHEHIYNQRRYMRSELTAFWRATSEEDMAQDTIIYTDESFTPDLNIFQDVLHRDTLVKAFLDQVFQLKPGLSLRSTFLAQFLLVLHRKALTLIKYIEDDTQKGKKPFKSLRNLKIDLDLTAEGDLNIIMALAEKIKPGLHSFIFGRPFYTSVQERDVLMTF

SEQ ID NO: 14 - DNA, 3356 bp, Homo sapiens
acgtaacctacggtgtcccgctaggaaagagaggtgcgtcaaacagcgacaagttccgcccacgtaaaagatgacgcttggtgtgtcagccgtccctgctgcccggttgcttctcttttgggggcggggtctagcaagagcaggtgtgggtttaggagatatctccggagcatttggataatgtgacagttggaatgcagtgatgtcgactctttgcccaccgccatctccagctgttgccaagacagagattgctttaagtggcaaatcacctttattagcagctacttttgcttactgggacaatattcttggtcctagagtaaggcacatttgggctccaaagacagaacaggtacttctcagtgatggagaaataacttttcttgccaaccacactctaaatggagaaatccttcgaaatgcagagagtggtgctatagatgtaaagttttttgtcttgtctgaaaagggagtgattattgtttcattaatctttgatggaaactggaatggggatcgcagcacatatggactatcaattatacttccacagacagaacttagtttctacctcccacttcatagagtgtgtgttgatagattaacacatataatccggaaaggaagaatatggatgcataaggaaagacaagaaaatgtccagaagattatcttagaaggcacagagagaatggaagatcagggtcagagtattattccaatgcttactggagaagtgattcctgtaatggaactgctttcatctatgaaatcacacagtgttcctgaagaaatagatatagctgatacagtactcaatgatgatgatattggtgacagctgtcatgaaggctttcttctcaatgccatcagctcacacttgcaaacctgtggctgttccgttgtagtaggtagcagtgcagagaaagtaaataagatagtcagaacattatgcctttttctgactccagcagagagaaaatgctccaggttatgtgaagcagaatcatcatttaaatatgagtcagggctctttgtacaaggcctgctaaaggattcaactggaagctttgtgctgcctttccggcaagtcatgtatgctccatatcccaccacacacatagatgtggatgtcaatactgtgaagcagatgccaccctgtcatgaacatatttataatcagcgtagatacatgagatccgagctgacagccttctggagagccacttcagaagaagacatggctcaggatacgatcatctacactgacgaaagctttactcctgatttgaatatttttcaagatgtcttacacagagacactctagtgaaagccttcctggatcaggtctttcagctgaaacctggcttatctctcagaagtactttccttgcacagtttctacttgtccttcacagaaaagccttgacactaataaaatatatagaagacgatacgcagaagggaaaaaagccctttaaatctcttcggaacctgaagatagaccttgatttaacagcagagggcgatcttaacataataatggctctggctgagaaaattaaaccaggcctacactcttttatctttggaagacctttctacactagtgtgcaagaacgagatgttctaatgactttttaaatgtgtaacttaataagcctattccatcacaatcatgatcgctggtaaagtagctcagtggtgtggggaaacgttcccctggatcatactccagaattctgctctcagcaattgcagttaagtaagttacactacagttctcacaagagcctgtgaggggatgtcaggtgcatcattacattgggtgtctcttttcctagatttatgcttttgggatacagacctatgtttacaatataataaatattattgctatcttttaaagatataataataggatgtaaacttgaccacaactactgtttttttgaaatacatgattcatggtttacatgtgtcaaggtgaaatctgagttggcttttacagatagttgactttctatcttttggcattctttggtgtgtagaattactgtaatacttctgcaatcaactgaaaactagagcctttaaatgatttcaattccacagaaagaaagtgagcttgaacataggatgagctttagaaagaaaattgatcaagcagatgtttaattggaattgattattagatcctactttgtggatttagtccctgggattcagtctgtagaaatgtctaatagttctctatagtccttgttcctggtgaaccacagttagggtgttttgtttattttattgttcttgctattgttgatattctatgtagttgagctctgtaaaaggaaattgtattttatgttttagtaattgttgccaactttttaaattaattttcattatttttgagccaaattgaaatgtgcacctcctgtgccttttttctccttagaaaatctaattacttggaacaagttcagatttcactggtcagtcattttcatcttgttttcttcttgctaagtcttaccatgtacctgctttggcaatcattgcaactctgagattataaaatgccttagagaatatactaactaataagatctttttttcagaaacagaaaatagttccttgagtacttccttcttgcatttctgcctatgtttttgaagttgttgctgtttgcctgcaataggctataaggaatagcaggagaaattttactgaagtgctgttttcctaggtgctactttggcagagctaagttatcttttgttttcttaatgcgtttggaccattttgctggctataaaataactgattaatataattctaacacaatgttgacattgtagttacacaaacacaaataaatattttatttaaaattctggaagtaatataaaagggaaaatatatttataagaaagggataaaggtaatagagcccttctgccccccacccaccaaatttacacaacaaaatgacatgttcgaatgtgaaaggtcataatagctttcccatcatgaatcagaaagatgtggacagcttgatgttttagacaaccactgaactagatgactgttgtactgtagctcagtcatttaaaaaatatataaatactaccttgtagtgtcccatactgtgttttttacatggtagattcttatttaagtgctaactggttattttctttggctggtttattgtactgttatacagaatgtaagttgtacagtgaaataagttattaaagcatgtgtaaacattgttatatatcttttctcctaaatggagaattttgaataaaatatatttgaaattttaaaaaaaaaaaaaaaaaa

SEQ ID NO: 15 - protein, 481 aa, Homo sapiens; identical to SEQ ID NO: 13

SEQ ID NO: 16 - DNA, 3198 bp, Mus musculus
gtgtccggggcggggcggtcccggggcggggcccggagcgggctgcggttgcggtccctgcgccggcggtgaaggcgcagcagcggcgagtggctattgcaagcgttcggataatgtgagacctggaatgcagtgagacctgggatgcagggatgtcgactatctgccccccaccatctcctgctgttgccaagacagagattgctttaagtggtgaatcacccttgttggcggctacctttgcttactgggataatattcttggtcctagagtaaggcatatttgggctccaaagacagaccaagtgcttctcagtgatggagaaataacttttcttgccaaccacactctaaatggagaaattcttcgaaatgcagagagtggggctatagatgtaaaattttttgtcttatctgaaaaaggggtaattattgtttcattaatcttcgacggaaactggaatggagatcggagcacttatggactatcaattatactgccgcagacagagctgagcttctacctcccacttcacagagtgtgtgttgacaggctaacacacattattcgaaaaggaagaatatggatgcataaggaaagacaagaaaatgtccagaaaattgtcttggaaggcacagagaggatggaagatcagggtcagagtatcattcccatgcttactggggaagtcattcctgtaatggagctgcttgcatctatgaaatcccacagtgttcctgaagacattgatatagctgatacagtgctcaatgatgatgacattggtgacagctgtcacgaaggctttcttctcaatgccatcagctcacacctgcagacctgtggctgttccgttgtagttggcagcagtgcagagaaagtaaataagatagtaagaacgctgtgcctttttctgacaccagcagagaggaaatgctccaggctgtgtgaagcagaatcgtcctttaagtacgaatcgggactctttgtgcaaggcttgctaaaggatgcaacaggcagttttgtcctacccttccggcaagttatgtatgccccgtaccccaccacgcacattgatgtggatgtcaacactgtcaagcagatgccaccgtgtcatgaacatatttataatcaacgcagatacatgaggtcagagctgacagccttctggagggcaacttcagaagaggacatggcgcaggacaccatcatctacacagatgagagcttcactcctgatttgaatattttccaagatgtcttacacagagacactctagtgaaagccttcctggatcaggtcttccatttgaagcctggcctgtctctcaggagtactttccttgcacagttcctcctcattcttcacagaaaagccttgacactaatcaagtacatcgaggatgatacgcagaaggggaaaaagccctttaagtctcttcggaacctgaagatagatcttgatttaacagcagagggcgatcttaacataataatggctctagctgagaaaattaagccaggcctacactctttcatctttgggagacctttctacactagtgtacaagaacgtgatgttctaatgaccttttgaccgtgtggtttgctgtgtctgtctcttcacagtcacacctgctgttacagtgtctcagcagtgtgtgggcacatccttcctcccgagtcctgctgcaggacagggtacactacacttgtcagtagaagtctgtacctgatgtcaggtgcatcgttacagtgaatgactcttcctagaatagatgtactcttttagggccttatgtttacaattatcctaagtactattgctgtcttttaaagatatgaatgatggaatatacacttgaccataactgctgattggttttttgttttgttttgtttgttttcttggaaacttatgattcctggtttacatgtaccacactgaaaccctcgttagctttacagataaagtgtgagttgacttcctgcccctctgtgttctgtggtatgtccgattacttctgccacagctaaacattagagcatttaaagtttgcagttcctcagaaaggaacttagtctgactacagattagttcttgagagaagacactgatagggcagagctgtaggtgaaatcagttgttagcccttcctttatagacgtagtccttcagattcggtctgtacagaaatgccgaggggtcatgcatgggccctgagtatcgtgacctgtgacaagttttttgttggtttattgtagttctgtcaaagaaagtggcatttgtttttataattgttgccaacttttaaggttaattttcattatttttgagccgaattaaaatgcgcacctcctgtgcctttcccaatcttggaaaatataatttcttggcagagggtcagatttcagggcccagtcactttcatctgaccaccctttgcacggctgccgtgtgcctggcttagattagaagtccttgttaagtatgtcagagtacattcgctgataagatctttgaagagcagggaagcgtcttgcctctttcctttggtttctgcctgtactctggtgtttcccgtgtcacctgcatcataggaacagcagagaaatctgacccagtgctatttttctaggtgctactatggcaaactcaagtggtctgtttctgttcctgtaacgttcgactatctcgctagctgtgaagtactgattagtggagttctgtgcaacagcagtgtaggagtatacacaaacacaaatatgtgtttctatttaaaactgtggacttagcataaaaagggagaatatatttattttttacaaaagggataaaaatgggccccgttcctcacccaccagatttagcgagaaaaagctttctattctgaaaggtcacggtggctttggcattacaaatcagaacaacacacactgaccatgatggcttgtgaactaactgcaaggcactccgtcatggtaagcgagtaggtcccacctcctagtgtgccgctcattgctttacacagtagaatcttatttgagtgctaattgttgtctttgctgctttactgtgttgttatagaaaatgtaagctgtacagtgaataagttattgaagcatgtgtaaacactgttatatatcttttctcctagatggggaattttgaataaaatacctttgaaattctgtgt

SEQ ID NO: 17 - protein, 481 aa, Mus musculus
MSTICPPPSPAVAKTEIALSGESPLLAATFAYWDNILGPRVRHIWAPKTDQVLLSDGEITFLANHTLNGEILRNAESGAIDVKFFVLSEKGVIIVSLIFDGNWNGDRSTYGLSIILPQTELSFYLPLHRVCVDRLTHIIRKGRIWMHKERQENVQKIVLEGTERMEDQGQSIIPMLTGEVIPVMELLASMKSHSVPEDIDIADTVLNDDDIGDSCHEGFLLNAISSHLQTCGCSVVVGSSAEKVNKIVRTLCLFLTPAERKCSRLCEAESSFKYESGLFVQGLLKDATGSFVLPFRQVMYAPYPTTHIDVDVNTVKQMPPCHEHIYNQRRYMRSELTAFWRATSEEDMAQDTIIYTDESFTPDLNIFQDVLHRDTLVKAFLDQVFHLKPGLSLRSTFLAQFLLILHRKALTLIKYIEDDTQKGKKPFKSLRNLKIDLDLTAEGDLNIIMALAEKIKPGLHSFIFGRPFYTSVQERDVLMTF

SEQ ID NO: 18 - DNA, 3435 bp, Rattus norvegicus
cgtttgtagtgtcagccatcccaattgcctgttccttctctgtgggagtggtgtctagacagtccaggcagggtatgctaggcaggtgcgttttggttgcctcagatcgcaacttgactccataacggtgaccaaagacaaaagaaggaaaccagattaaaaagaaccggacacagacccctgcagaatctggagcggccgtggttgggggcggggctacgacggggcggactcgggggcgtgggagggcggggccggggcggggcccggagccggctgcggttgcggtccctgcgccggcggtgaaggcgcagcggcggcgagtggctattgcaagcgtttggataatgtgagacctgggatgcagggatgtcgactatctgccccccaccatctcctgctgttgccaagacagagattgctttaagtggtgaatcacccttgttggcggctacctttgcttactgggataatattcttggtcctagagtaaggcacatttgggctccaaagacagaccaagtactcctcagtgatggagaaatcacttttcttgccaaccacactctgaatggagaaattcttcggaatgcggagagtggggcaatagatgtaaagttttttgtcttatctgaaaagggcgtcattattgtttcattaatcttcgacgggaactggaacggagatcggagcacttacggactatcaattatactgccgcagacggagctgagtttctacctcccactgcacagagtgtgtgttgacaggctaacgcacatcattcgaaaaggaaggatatggatgcacaaggaaagacaagaaaatgtccagaaaattgtcttggaaggcaccgagaggatggaagatcagggtcagagtatcatccctatgcttactggggaggtcatccctgtgatggagctgcttgcgtctatgagatcacacagtgttcctgaagacctcgatatagctgatacagtactcaatgatgatgacattggtgacagctgtcatgaaggctttcttctcaatgccatcagctcacatctgcagacctgcggctgttctgtggtggtaggcagcagtgcagagaaagtaaataagatagtaagaacactgtgcctttttctgacaccagcagagaggaagtgctccaggctgtgtgaagccgaatcgtcctttaaatacgaatctggactctttgtacaaggcttgctaaaggatgcgactggcagttttgtactacctttccggcaagttatgtatgccccttatcccaccacacacatcgatgtggatgtcaacactgtcaagcagatgccaccgtgtcatgaacatatttataatcaacgcagatacatgaggtcagagctgacagccttctggagggcaacttcagaagaggacatggctcaggacaccatcatctacacagatgagagcttcactcctgatttgaatattttccaagatgtcttacacagagacactctagtgaaagcctttctggatcaggtcttccatttgaagcctggcctgtctctcaggagtactttccttgcacagttcctcctcattcttcacagaaaagccttgacactaatcaagtacatagaggatgacacgcagaaggggaaaaagccctttaagtctcttcggaacctgaagatagatcttgatttaacagcagagggcgaccttaacataataatggctctagctgagaaaattaagccaggcctacactctttcatcttcgggagacctttctacactagtgtccaagaacgtgatgttctaatgactttttaaacatgtggtttgctccgtgtgtctcatgacagtcacacttgctgttacagtgtctcagcgctttggacacatccttcctccagggtcctgccgcaggacacgttacactacacttgtcagtagaggtctgtaccagatgtcaggtacatcgttgtagtgaatgtctcttttcctagactagatgtaccctcgtagggacttatgtttacaaccctcctaagtactagtgctgtcttgtaaggatacgaatgaagggatgtaaacttcaccacaactgctggttggttttgttgtttttgttttttgaaacttataattcatggtttacatgcatcacactgaaaccctagttagctttttacaggtaagctgtgagttgactgcctgtccctgtgttctctggcctgtacgatctgtggcgtgtaggatcacttttgcaacaactaaaaactaaagcactttgtttgcagttctacagaaagcaacttagtctgtctgcagattcgtttttgaaagaagacatgagaaagcggagttttaggtgaagtcagttgttggatcttcctttatagacttagtcctttagatgtggtctgtatagacatgcccaaccatcatgcatgggcactgaatatcgtgaactgtggtatgctttttgttggtttattgtacttctgtcaaagaaagtggcattggtttttataattgttgccaagttttaaggttaattttcattatttttgagccaaattaaaatgtgcacctcctgtgcctttcccaatcttggaaaatataatttcttggcagaaggtcagatttcagggcccagtcactttcgtctgacttccctttgcacagtccgccatgggcctggcttagaagttcttgtaaactatgccagagagtacattcgctgataaaatcttctttgcagagcaggagagcttcttgcctctttcctttcatttctgcctggactttggtgttctccacgttccctgcatcctaaggacagcaggagaactctgaccccagtgctatttctctaggtgctattgtggcaaactcaagcggtccgtctctgtccctgtaacgttcgtaccttgctggctgtgaagtactgactggtaaagctccgtgctacagcagtgtagggtatacacaaacacaagtaagtgttttatttaaaactgtggacttagcataaaaagggagactatatttattttttacaaaagggataaaaatggaaccctttcctcacccaccagatttagtcagaaaaaaacattctattctgaaaggtcacagtggttttgacatgacacatcagaacaacgcacactgtccatgatggcttatgaactccaagtcactccatcatggtaaatgggtagatccctccttctagtgtgccacaccattgcttcccacagtagaatcttatttaagtgctaagtgttgtctctgctggtttactctgttgttttagagaatgtaagttgtatagtgaataagttattgaagcatgtgtaaacactgttatacatcttttctcctagatggggaatttggaataaaatacctttaaaattcaaaaaaaaaaaaaaaaaaaaaaaa

SEQ ID NO: 19 - protein, 481 aa, Rattus norvegicus
MSTICPPPSPAVAKTEIALSGESPLLAATFAYWDNILGPRVRHIWAPKTDQVLLSDGEITFLANHTLNGEILRNAESGAIDVKFFVLSEKGVIIVSLIFDGNWNGDRSTYGLSIILPQTELSFYLPLHRVCVDRLTHIIRKGRIWMHKERQENVQKIVLEGTERMEDQGQSIIPMLTGEVIPVMELLASMRSHSVPEDLDIADTVLNDDDIGDSCHEGFLLNAISSHLQTCGCSVVVGSSAEKVNKIVRTLCLFLTPAERKCSRLCEAESSFKYESGLFVQGLLKDATGSFVLPFRQVMYAPYPTTHIDVDVNTVKQMPPCHEHIYNQRRYMRSELTAFWRATSEEDMAQDTIIYTDESFTPDLNIFQDVLHRDTLVKAFLDQVFHLKPGLSLRSTFLAQFLLILHRKALTLIKYIEDDTQKGKKPFKSLRNLKIDLDLTAEGDLNIIMALAEKIKPGLHSFIFGRPFYTSVQERDVLMTF

SEQ ID NO: 20 - DNA, 100 bp, Mus musculus
gaaccgcggcgcgtcaagcagagacgagttccgcccacgtgaaagatggcgtttgtagtgacagccatcccaattgccctttccttctaggtggaaagtg

SEQ ID NO: 21 - DNA, 2648 bp, Artificial Sequence
  floxed neo cassette of 8026 plus lox sites
ataacttcgtataatgtatgctatacgaagttatatgcatggcctccgcgccgggttttggcgcctcccgcgggcgcccccctcctcacggcgagcgctgccacgtcagacgaagggcgcagcgagcgtcctgatccttccgcccggacgctcaggacagcggcccgctgctcataagactcggccttagaaccccagtatcagcagaaggacattttaggacgggacttgggtgactctagggcactggttttctttccagagagcggaacaggcgaggaaaagtagtcccttctcggcgattctgcggagggatctccgtggggcggtgaacgccgatgattatataaggacgcgccgggtgtggcacagctagttccgtcgcagccgggatttgggtcgcggttcttgtttgtggatcgctgtgatcgtcacttggtgagtagcgggctgctgggctggccggggctttcgtggccgccgggccgctcggtgggacggaagcgtgtggagagaccgccaagggctgtagtctgggtccgcgagcaaggttgccctgaactgggggttggggggagcgcagcaaaatggcggctgttcccgagtcttgaatggaagacgcttgtgaggcgggctgtgaggtcgttgaaacaaggtggggggcatggtgggcggcaagaacccaaggtcttgaggccttcgctaatgcgggaaagctcttattcgggtgagatgggctggggcaccatctggggaccctgacgtgaagtttgtcactgactggagaactcggtttgtcgtctgttgcgggggcggcagttatggcggtgccgttgggcagtgcacccgtacctttgggagcgcgcgccctcgtcgtgtcgtgacgtcacccgttctgttggcttataatgcagggtggggccacctgccggtaggtgtgcggtaggcttttctccgtcgcaggacgcagggttcgggcctagggtaggctctcctgaatcgacaggcgccggacctctggtgaggggagggataagtgaggcgtcagtttctttggtcggttttatgtacctatcttcttaagtagctgaagctccggttttgaactatgcgctcggggttggcgagtgtgttttgtgaagttttttaggcaccttttgaaatgtaatcatttgggtcaatatgtaattttcagtgttagactagtaaattgtccgctaaattctggccgtttttggcttttttgttagacgtgttgacaattaatcatcggcatagtatatcggcatagtataatacgacaaggtgaggaactaaaccatgggatcggccattgaacaagatggattgcacgcaggttctccggccgcttgggtggagaggctattcggctatgactgggcacaacagacaatcggctgctctgatgccgccgtgttccggctgtcagcgcaggggcgcccggttctttttgtcaagaccgacctgtccggtgccctgaatgaactgcaggacgaggcagcgcggctatcgtggctggccacgacgggcgttccttgcgcagctgtgctcgacgttgtcactgaagcgggaagggactggctgctattgggcgaagtgccggggcaggatctcctgtcatctcaccttgctcctgccgagaaagtatccatcatggctgatgcaatgcggcggctgcatacgcttgatccggctacctgcccattcgaccaccaagcgaaacatcgcatcgagcgagcacgtactcggatggaagccggtcttgtcgatcaggatgatctggacgaagagcatcaggggctcgcgccagccgaactgttcgccaggctcaaggcgcgcatgcccgacggcgatgatctcgtcgtgacccatggcgatgcctgcttgccgaatatcatggtggaaaatggccgcttttctggattcatcgactgtggccggctgggtgtggcggaccgctatcaggacatagcgttggctacccgtgatattgctgaagagcttggcggcgaatgggctgaccgcttcctcgtgctttacggtatcgccgctcccgattcgcagcgcatcgccttctatcgccttcttgacgagttcttctgaggggatccgctgtaagtctgcagaaattgatgatctattaaacaataaagatgtccactaaaatggaagtttttcctgtcatactttgttaagaagggtgagaacagagtacctacattttgaatggaaggattggagctacgggggtgggggtggggtgggattagataaatgcctgctctttactgaaggctctttactattgctttatgataatgtttcatagttggatatcataatttaaacaagcaaaaccaaattaagggccagctcattcctcccactcatgatctatagatctatagatctctcgtgggatcattgtttttctcttgattcccactttgtggttctaagtactgtggtttccaaatgtgtcagtttcatagcctgaagaacgagatcagcagcctctgttccacatacacttcattctcagtattgttttgccaagttctaattccatcagacctcgacctgcagcccctagataacttcgtataatgtatgctatacgaagttat

SEQ ID NO: 22 - DNA, 100 bp, Mus musculus
attgtgacttgggcatcacttgactgatggtaatcagttgcagagagagaagtgcactgattaagtctgtccacacagggtctgtctggccaggagtgca

SEQ ID NO: 23 - DNA, 100 bp, Mus musculus; identical to SEQ ID NO: 20

SEQ ID NO: 24 - DNA, 2648 bp, Artificial Sequence; identical to SEQ ID NO: 21
  floxed cassette of 8028 plus lox sites

SEQ ID NO: 25 - DNA, 100 bp, Mus musculus; identical to SEQ ID NO: 22

SEQ ID NO: 26 - DNA, 680 bp, Mus musculus
ccagtagcagcacccacgtccaccttctgtctagtaatgtccaacacctccctcagtccaaacactgctctgcatccatgtggctcccatttatacctgaagcacttgatggggcctcaatgttttactagagcccacccccctgcaactctgagaccctctggatttgtctgtcagtgcctcactggggcgttggataatttcttaaaaggtcaagttccctcagcagcattctctgagcagtctgaagatgtgtgcttttcacagttcaaatccatgtggctgtttcacccacctgcctggccttgggttatctatcaggacctagcctagaagcaggtgtgtggcacttaacacctaagctgagtgactaactgaacactcaagtggatgccatctttgtcacttcttgactgtgacacaagcaactcctgatgccaaagccctgcccacccctctcatgcccatatttggacatggtacaggtcctcactggccatggtctgtgaggtcctggtcctctttgacttcataattcctaggggccactagtatctataagaggaagagggtgctggctcccaggccacagcccacaaaattccacctgctcacaggttggctggctcgacccaggtggtgtcccctgctctgagccagctcccggccaagccagcacc

SEQ ID NO: 27 - DNA, 1052 bp, Mus musculus
tgccatcatcacaggatgtccttccttctccagaagacagactggggctgaaggaaaagccggccaggctcagaacgagccccactaattactgcctccaacagctttccactcactgcccccagcccaacatcccctttttaactgggaagcattcctactctccattgtacgcacacgctcggaagcctggctgtgggtttgggcatgagaggcagggacaacaaaaccagtatatatgattataactttttcctgtttccctatttccaaatggtcgaaaggaggaagttaggtctacctaagctgaatgtattcagttagcaggagaaatgaaatcctatacgtttaatactagaggagaaccgccttagaatatttatttcattggcaatgactccaggactacacagcgaaattgtattgcatgtgctgccaaaatactttagctctttccttcgaagtacgtcggatcctgtaattgagacaccgagtttaggtgactagggttttcttttgaggaggagtcccccaccccgccccgctctgccgcgacaggaagctagcgatccggaggacttagaatacaatcgtagtgtgggtaaacatggagggcaagcgcctgcaaagggaagtaagaagattcccagtccttgttgaaatccatttgcaaacagaggaagctgccgcgggtcgcagtcggtggggggaagccctgaaccccacgctgcacggctgggctggccaggtgcggccacgcccccatcgcggcggctggtaggagtgaatcagaccgtcagtattggtaaagaagtctgcggcagggcagggagggggaagagtagtcagtcgctcgctcactcgctcgctcgcacagacactgctgcagtgacactcggccctccagtgtcgcggagacgcaagagcagcgcgcagcacctgtccgcccggagcgagcccggcccgcggccgtagaaaaggagggaccgccgaggtgcgcgtcagtactgctcagcccggcagggacgcgggaggatgtggactgggtggac

SEQ ID NO: 28 - DNA, 2008 bp, Mus musculus
gtggtgctgactcagcatcggttaataaaccctctgcaggaggctggatttcttttgtttaattatcacttggacctttctgagaactcttaagaattgttcattcgggtttttttgttttgttttggtttggtttttttgggttttttttttttttttttttttggtttttggagacagggtttctctgtatatagccctggcacaagagcaagctaacagcctgtttcttcttggtgctagcgccccctctggcagaaaatgaaataacaggtggacctacaacccccccccccccccccagtgtattctactcttgtccccggtataaatttgattgttccgaactacataaattgtagaaggattttttagatgcacatatcattttctgtgataccttccacacacccctcccccccaaaaaaatttttctgggaaagtttcttgaaaggaaaacagaagaacaagcctgtctttatgattgagttgggcttttgttttgctgtgtttcatttcttcctgtaaacaaatactcaaatgtccacttcattgtatgactaagttggtatcattaggttgggtctgggtgtgtgaatgtgggtgtggatctggatgtgggtgggtgtgtatgccccgtgtgtttagaatactagaaaagataccacatcgtaaacttttgggagagatgatttttaaaaatgggggtgggggtgaggggaacctgcgatgaggcaagcaagataaggggaagacttgagtttctgtgatctaaaaagtcgctgtgatgggatgctggctataaatgggcccttagcagcattgtttctgtgaattggaggatccctgctgaaggcaaaagaccattgaaggaagtaccgcatctggtttgttttgtaatgagaagcaggaatgcaaggtccacgctcttaataataaacaaacaggacattgtatgccatcatcacaggatgtccttccttctccagaagacagactggggctgaaggaaaagccggccaggctcagaacgagccccactaattactgcctccaacagctttccactcactgcccccagcccaacatcccctttttaactgggaagcattcctactctccattgtacgcacacgctcggaagcctggctgtgggtttgggcatgagaggcagggacaacaaaaccagtatatatgattataactttttcctgtttccctatttccaaatggtcgaaaggaggaagttaggtctacctaagctgaatgtattcagttagcaggagaaatgaaatcctatacgtttaatactagaggagaaccgccttagaatatttatttcattggcaatgactccaggactacacagcgaaattgtattgcatgtgctgccaaaatactttagctctttccttcgaagtacgtcggatcctgtaattgagacaccgagtttaggtgactagggttttcttttgaggaggagtcccccaccccgccccgctctgccgcgacaggaagctagcgatccggaggacttagaatacaatcgtagtgtgggtaaacatggagggcaagcgcctgcaaagggaagtaagaagattcccagtccttgttgaaatccatttgcaaacagaggaagctgccgcgggtcgcagtcggtggggggaagccctgaaccccacgctgcacggctgggctggccaggtgcggccacgcccccatcgcggcggctggtaggagtgaatcagaccgtcagtattggtaaagaagtctgcggcagggcagggagggggaagagtagtcagtcgctcgctcactcgctcgctcgcacagacactgctgcagtgacactcggccctccagtgtcgcggagacgcaagagcagcgcgcagcacctgtccgcccggagcgagcccggcccgcggccgtagaaaaggagggaccgccgaggtgcgcgtcagtactgctcagcccggcagggacgcgggaggatgtggactgggtggac

SEQ ID NO: 29 - DNA, 252 bp, Artificial Sequence
  Southern blot probe
ccggggcggggctgcggttgcggtgcctgcgcccgcggcggcggaggcgcaggcggtggcgagtgggtgagtgaggaggcggcatcctggcgggtggctgtttggggttcggctgccgggaagaggcgcgggtagaagcgggggctctcctcagagctcgacgcatttttactttccctctcatttctctgaccgaagctgggtgtcgggctttcgcctctagcgactggtggaattgcctgcatccgggcc

SEQ ID NO: 30 - DNA, 39 bp, Artificial Sequence
  Asuragen 2-Primer Fwd
tgcgcctccgccgccgcgggcgcaggcaccgcaaccgca

SEQ ID NO: 31 - DNA, 35 bp, Artificial Sequence
  Asuragen 2-Primer Rev
cgcagcctgtagcaagctctggaactcaggagtcg

SEQ ID NO: 32 - DNA, 36 bp, Artificial Sequence
  Asuragen 3-Primer Fwd
atgcaggcaattccaccagtcgctagaggcgaaagc

SEQ ID NO: 33 - DNA, 40 bp, Artificial Sequence
  Asuragen 3-Primer Rev
taaccagaagaaaacaaggagggaaacaaccgcagcctgt

SEQ ID NO: 34 - DNA, 158 bp, Homo sapiens
acgtaacctacggtgtcccgctaggaaagagaggtgcgtcaaacagcgacaagttccgcccacgtaaaagatgacgcttggtgtgtcagccgtccctgctgcccggttgcttctcttttgggggcggggtctagcaagagcaggtgtgggtttaggag

SEQ ID NO: 35 - DNA, 487 bp, Homo sapiens
tatctccggagcatttggataatgtgacagttggaatgcagtgatgtcgactctttgcccaccgccatctccagctgttgccaagacagagattgctttaagtggcaaatcacctttattagcagctacttttgcttactgggacaatattcttggtcctagagtaaggcacatttgggctccaaagacagaacaggtacttctcagtgatggagaaataacttttcttgccaaccacactctaaatggagaaatccttcgaaatgcagagagtggtgctatagatgtaaagttttttgtcttgtctgaaaagggagtgattattgtttcattaatctttgatggaaactggaatggggatcgcagcacatatggactatcaattatacttccacagacagaacttagtttctacctcccacttcatagagtgtgtgttgatagattaacacatataatccggaaaggaagaatatggatgcataag

SEQ ID NO: 36 - DNA, 198 bp, Homo sapiens
gggtctagcaagagcaggtgtgggtttaggaggtgtgtgtttttgtttttcccaccctctctccccactacttgctctcacagtactcgctgagggtgaacaagaaaagacctgataaagattaaccagaagaaaacaaggagggaaacaaccgcagcctgtagcaagctctggaactcaggagtcgcgcgctatgcg

SEQ ID NO: 37 - DNA, 118 bp, Homo sapiens
gcgatcgcggggcgtggtcggggcgggcccgggggcgggcccggggcggggctgcggttgcggtgcctgcgcccgcggcggcggaggcgcaggcggtggcgagtgggtgagtgaggag

SEQ ID NO: 38 - DNA, 20 bp, Artificial Sequence
  Synthetic
agtactgtgagagcaagtag

SEQ ID NO: 39 - DNA, 20 bp, Artificial Sequence
  Synthetic
gctctcacagtactcgctga

SEQ ID NO: 40 - DNA, 20 bp, Artificial Sequence
  Synthetic
ccgcagcctgtagcaagctc

SEQ ID NO: 41 - DNA, 20 bp, Artificial Sequence
  Synthetic
cggccgctagcgcgatcgcg

SEQ ID NO: 42 - DNA, 20 bp, Artificial Sequence
  Synthetic
acgccccgcgatcgcgctag

SEQ ID NO: 43 - DNA, 20 bp, Artificial Sequence
  Synthetic
tggcgagtgggtgagtgagg

SEQ ID NO: 44 - DNA, 20 bp, Artificial Sequence
  Synthetic
ggaagaggcgcgggtagaag

SEQ ID NO: 45 - DNA, 1302 bp, Artificial Sequence
  Synthetic
gaacttacggagtcccacgagggaaccgcggcgcgtcaagcagagacgagttccgcccacgtgaaagatggcgtttgtagtgacagccatcccaattgccctttccttctaggtggaaagtggggtctagcaagagcaggtgtgggtttaggaggtgtgtgtttttgtttttcccaccctctctccccactacttgctctcacagtactcgctgagggtgaacaagaaaagacctgataaagattaaccagaagaaaacaaggagggaaacaaccgcagcctgtagcaagctctggaactcaggagtcgcgcgctatgcgatcgccgtctcggggccggggccggggccggggccggggccggggccggggccggggccggggccggggccggggccggggccggggccggggccggggccggggccggggccggggccggggccggggccggggccggggccggggccggggccggggccggggccggggccggggccggggccggggccggggccggggccggggccggggccggggccggggccggggccggggccggggccggggccggggccggggccggggccggggccggggccggggccggggccggggccggggccggggccggggccggggccggggccggggccggggccggggccggggccggggccggggccggggccggggccggggccggggccggggccggggccggggccggggccggggccggggccggggccggggccggggccggggccggggccggggccggggccggggccggggccggggccggggccggggccggggccggggccggggccggggccggggccggggccggggccggggccggggccggggccggggccgagaccctcgagggccggccgctagcgcgatcgcggggcgtggtcggggcgggcccgggggcgggcccggggcggggctgcggttgcggtgcctgcgcccgcggcggcggaggcgcaggcggtgcgagtgggtgagtgaggaggcggcatcctggcgggtggctgtttggggttcggctgccgggaagaggcgcgggtagaagcgggggctctcctcagagctcgacgcatttttactttccctctcatttctctgaccgaagctgggtgtcgggctttcgcctctagcgactggtggaattgcctgcatccgggccccgggcttcccggcggcggcggcggcggcggcggcgcagggacaagggatggggatctggcctcttccttgctttcccgccctcagtacccgagctgtctcc

SEQ ID NO: 46 - DNA, 21 bp, Artificial Sequence
  Synthetic
gagtactgtgagagcaagtag

SEQ ID NO: 47 - DNA, 21 bp, Artificial Sequence
  Synthetic
gccgcagcctgtagcaagctc

SEQ ID NO: 48 - DNA, 21 bp, Artificial Sequence
  Synthetic
gcggccgctagcgcgatcgcg

SEQ ID NO: 49 - DNA, 21 bp, Artificial Sequence
  Synthetic
gacgccccgcgatcgcgctag

SEQ ID NO: 50 - DNA, 21 bp, Artificial Sequence
  Synthetic
gtggcgagtgggtgagtgagg

SEQ ID NO: 51 - DNA, 26 bp, Artificial Sequence
  Synthetic
acaccgctctcacagtactcgctgag

SEQ ID NO: 52 - DNA, 27 bp, Artificial Sequence
  Synthetic
acaccgccgcagcctgtagcaagctcg

SEQ ID NO: 53 - DNA, 27 bp, Artificial Sequence
  Synthetic
acaccgagtactgtgagagcaagtagg

SEQ ID NO: 54 - DNA, 27 bp, Artificial Sequence
  Synthetic
acaccgacgccccgcgatcgcgctagg

SEQ ID NO: 55 - DNA, 27 bp, Artificial Sequence
  Synthetic
acaccgcggccgctagcgcgatcgcgg

SEQ ID NO: 56 - DNA, 27 bp, Artificial Sequence
  Synthetic
acaccgtggcgagtgggtgagtgaggg

SEQ ID NO: 57 - DNA, 26 bp, Artificial Sequence
  Synthetic
acaccggaagaggcgcgggtagaagg

SEQ ID NO: 58 - DNA, 20 bp, Artificial Sequence
  Synthetic
gacgcgttaatgccaacttt

SEQ ID NO: 59 - DNA, 20 bp, Artificial Sequence
  Synthetic
gagggcctatttcccatgat

SEQ ID NO: 60 - DNA, 20 bp, Artificial Sequence
  Synthetic
gacgcgttaatgccaacttt

SEQ ID NO: 61 - DNA, 20 bp, Artificial Sequence
  Synthetic
gaacttacggagtcccacga

SEQ ID NO: 62 - DNA, 20 bp, Artificial Sequence
  Synthetic
ggagacagctcgggtactga

SEQ ID NO: 63 - DNA, 82 bp, Artificial Sequence
  Synthetic
gttggaaccattcaaaacagcatagcaagttaaaataaggctagtccgttatcaacttgaaaaagtggcaccgagtcggtgc

SEQ ID NO: 64 - DNA, 76 bp, Artificial Sequence
  Synthetic
gttttagagctagaaatagcaagttaaaataaggctagtccgttatcaacttgaaaaagtggcaccgagtcggtgc

SEQ ID NO: 65 - DNA, 86 bp, Artificial Sequence
  Synthetic
gtttaagagctatgctggaaacagcatagcaagtttaaataaggctagtccgttatcaacttgaaaaagtggcaccgagtcggtgc

SEQ ID NO: 66 - DNA, 19 bp, Artificial Sequence
  Forward Primer
catcccaattgccctttcc

SEQ ID NO: 67 - DNA, 21 bp, Artificial Sequence
  Reverse Primer
cccacacctgctcttgctaga

SEQ ID NO: 68 - DNA, 17 bp, Artificial Sequence
  Probe
tctaggtggaaagtggg

SEQ ID NO: 69 - DNA, 20 bp, Artificial Sequence
  Forward Primer
gagcaggtgtgggtttagga

SEQ ID NO: 70 - DNA, 20 bp, Artificial Sequence
  Reverse Primer
ccaggtctcactgcattcca

SEQ ID NO: 71 - DNA, 26 bp, Artificial Sequence
  Probe
attgcaagcgttcggataatgtgaga

SEQ ID NO: 72 - DNA, 21 bp, Artificial Sequence
  Forward Primer
gctgtcacgaaggctttcttc

SEQ ID NO: 73 - DNA, 20 bp, Artificial Sequence
  Reverse Primer
gcactgctgccaactacaac

SEQ ID NO: 74 - DNA, 24 bp, Artificial Sequence
  Probe
tcaatgccatcagctcacacctgc

SEQ ID NO: 75 - DNA, 17 bp, Artificial Sequence
  Forward Primer
aagaggcgcgggtagaa

SEQ ID NO: 76 - DNA, 22 bp, Artificial Sequence
  Reverse Primer
cagcttcggtcagagaaatgag

SEQ ID NO: 77 - DNA, 24 bp, Artificial Sequence
  Probe
ctctcctcagagctcgacgcattt

SEQ ID NO: 78 - DNA, 20 bp, Artificial Sequence
  Forward Primer
ctgcacaatttcagcccaag

SEQ ID NO: 79 - DNA, 20 bp, Artificial Sequence
  Reverse Primer
caggtcatgtcccacagaat

SEQ ID NO: 80 - DNA, 24 bp, Artificial Sequence
  Probe
catatgagggcagcaatgcaagtc

SEQ ID NO: 81 - DNA, 16 bp, Artificial Sequence
  LNA Probe for sense G4C2 RNA
  TYE563 (1)..(1)
ccccggccccggcccc

SEQ ID NO: 82 - DNA, 22 bp, Artificial Sequence
  LNA Probe for antisense G4C2 RNA
  TYE563 (1)..(1)
ggggccggggccggggggcccc

SEQ ID NO: 83 - DNA, 18 bp, Artificial Sequence
  DNA Probe for sense G4C2 RNA
  Cy3 (18)..(18)
ccccggccccggccccgg

SEQ ID NO: 84 - DNA, 17 bp, Artificial Sequence
  DNA Probe for antisense G4C2 RNA
  Cy3 (17)..(17)
ggggccggggccggggc